European Patent Specification EP 3 431 494 B1, published May 1, 2024. Title: NERVE GROWTH FACTOR MUTANT. Applicant: STAIDSON(BEIJING) BIOPHARMACEUTICALS CO.,LTD. The sequence listing filed with the application follows.

SEQUENCE LISTING (42 sequences)

SEQ ID NO: 1 - DNA, 726 bp, Homo sapiens: DNA sequence of wild-type human NGF
atgtccatgttgttctacactctgatcacagcttttctgatcggcatacaggcggaaccacactcagagagcaatgtccctgcaggacacaccatcccccaagcccactggactaaacttcagcattcccttgacactgcccttcgcagagcccgcagcgccccggcagcggcgatagctgcacgcgtggcggggcagacccgcaacattactgtggaccccaggctgtttaaaaagcggcgactccgttcaccccgtgtgctgtttagcacccagcctccccgtgaagctgcagacactcaggatctggacttcgaggtcggtggtgctgcccccttcaacaggactcacaggagcaagcggtcatcatcccatcccatcttccacaggggcgaattctcggtgtgtgacagtgtcagcgtgtgggttggggataagaccaccgccacagacatcaagggcaaggaggtgatggtgttgggagaggtgaacattaacaacagtgtattcaaacagtacttttttgagaccaagtgccgggacccaaatcccgttgacagcgggtgccggggcattgactcaaagcactggaactcatattgtaccacgactcacacctttgtcaaggcgctgaccatggatggcaagcaggctgcctggcggtttatccggatagatacggcctgtgtgtgtgtgctcagcaggaaggctgtgagaagagcctga

SEQ ID NO: 2 - protein, 120 aa, Homo sapiens: amino acid sequence of wild-type human NGF
SSSHPIFHRGEFSVCDSVSVWVGDKTTATDIKGKEVMVLGEVNINNSVFKQYFFETKCRDPNPVDSGCRGIDSKHWNSYCTTTHTFVKALTMDGKQAAWRFIRIDTACVCVLSRKAVRRA

SEQ ID NO: 3 - protein, 120 aa, Homo sapiens NGF mutant Phe12Glu
SSSHPIFHRGEESVCDSVSVWVGDKTTATDIKGKEVMVLGEVNINNSVFKQYFFETKCRDPNPVDSGCRGIDSKHWNSYCTTTHTFVKALTMDGKQAAWRFIRIDTACVCVLSRKAVRRA

SEQ ID NO: 4 - protein, 120 aa, Homo sapiens NGF mutant Lys32Gly
SSSHPIFHRGEFSVCDSVSVWVGDKTTATDIGGKEVMVLGEVNINNSVFKQYFFETKCRDPNPVDSGCRGIDSKHWNSYCTTTHTFVKALTMDGKQAAWRFIRIDTACVCVLSRKAVRRA

SEQ ID NO: 5 - protein, 120 aa, Homo sapiens NGF mutant Lys32Leu
SSSHPIFHRGEFSVCDSVSVWVGDKTTATDILGKEVMVLGEVNINNSVFKQYFFETKCRDPNPVDSGCRGIDSKHWNSYCTTTHTFVKALTMDGKQAAWRFIRIDTACVCVLSRKAVRRA

SEQ ID NO: 6 - protein, 120 aa, Homo sapiens NGF mutant Lys32Tyr
SSSHPIFHRGEFSVCDSVSVWVGDKTTATDIYGKEVMVLGEVNINNSVFKQYFFETKCRDPNPVDSGCRGIDSKHWNSYCTTTHTFVKALTMDGKQAAWRFIRIDTACVCVLSRKAVRRA

SEQ ID NO: 7 - protein, 120 aa, Homo sapiens NGF mutant Arg59Leu
SSSHPIFHRGEFSVCDSVSVWVGDKTTATDIKGKEVMVLGEVNINNSVFKQYFFETKCLDPNPVDSGCRGIDSKHWNSYCTTTHTFVKALTMDGKQAAWRFIRIDTACVCVLSRKAVRRA

SEQ ID NO: 8 - protein, 120 aa, Homo sapiens NGF mutant Arg59Ala
SSSHPIFHRGEFSVCDSVSVWVGDKTTATDIKGKEVMVLGEVNINNSVFKQYFFETKCADPNPVDSGCRGIDSKHWNSYCTTTHTFVKALTMDGKQAAWRFIRIDTACVCVLSRKAVRRA

SEQ ID NO: 9 - protein, 120 aa, Homo sapiens NGF mutant Asp65Ala
SSSHPIFHRGEFSVCDSVSVWVGDKTTATDIKGKEVMVLGEVNINNSVFKQYFFETKCRDPNPVASGCRGIDSKHWNSYCTTTHTFVKALTMDGKQAAWRFIRIDTACVCVLSRKAVRRA

SEQ ID NO: 10 - protein, 120 aa, Homo sapiens NGF mutant Asp65Gly
SSSHPIFHRGEFSVCDSVSVWVGDKTTATDIKGKEVMVLGEVNINNSVFKQYFFETKCRDPNPVGSGCRGIDSKHWNSYCTTTHTFVKALTMDGKQAAWRFIRIDTACVCVLSRKAVRRA

SEQ ID NO: 11 - protein, 120 aa, Homo sapiens NGF mutant Lys74Leu
SSSHPIFHRGEFSVCDSVSVWVGDKTTATDIKGKEVMVLGEVNINNSVFKQYFFETKCRDPNPVDSGCRGIDSLHWNSYCTTTHTFVKALTMDGKQAAWRFIRIDTACVCVLSRKAVRRA

SEQ ID NO: 12 - protein, 120 aa, Homo sapiens NGF mutant Lys88Phe
SSSHPIFHRGEFSVCDSVSVWVGDKTTATDIKGKEVMVLGEVNINNSVFKQYFFETKCRDPNPVDSGCRGIDSKHWNSYCTTTHTFVFALTMDGKQAAWRFIRIDTACVCVLSRKAVRRA

SEQ ID NO: 13 - protein, 120 aa, Homo sapiens NGF mutant Lys88Leu
SSSHPIFHRGEFSVCDSVSVWVGDKTTATDIKGKEVMVLGEVNINNSVFKQYFFETKCRDPNPVDSGCRGIDSKHWNSYCTTTHTFVLALTMDGKQAAWRFIRIDTACVCVLSRKAVRRA

SEQ ID NO: 14 - protein, 120 aa, Homo sapiens NGF mutant Lys88Glu
SSSHPIFHRGEFSVCDSVSVWVGDKTTATDIKGKEVMVLGEVNINNSVFKQYFFETKCRDPNPVDSGCRGIDSKHWNSYCTTTHTFVEALTMDGKQAAWRFIRIDTACVCVLSRKAVRRA

SEQ ID NO: 15 - protein, 120 aa, Homo sapiens NGF mutant Lys88Gly
SSSHPIFHRGEFSVCDSVSVWVGDKTTATDIKGKEVMVLGEVNINNSVFKQYFFETKCRDPNPVDSGCRGIDSKHWNSYCTTTHTFVGALTMDGKQAAWRFIRIDTACVCVLSRKAVRRA

SEQ ID NO: 16 - protein, 120 aa, Homo sapiens NGF mutant Gln96Glu
SSSHPIFHRGEFSVCDSVSVWVGDKTTATDIKGKEVMVLGEVNINNSVFKQYFFETKCRDPNPVDSGCRGIDSKHWNSYCTTTHTFVKALTMDGKEAAWRFIRIDTACVCVLSRKAVRRA

SEQ ID NO: 17 - protein, 120 aa, Homo sapiens NGF mutant Arg114Val
SSSHPIFHRGEFSVCDSVSVWVGDKTTATDIKGKEVMVLGEVNINNSVFKQYFFETKCRDPNPVDSGCRGIDSKHWNSYCTTTHTFVKALTMDGKQAAWRFIRIDTACVCVLSVKAVRRA

SEQ ID NO: 18 - protein, 120 aa, Homo sapiens NGF mutant Arg114Phe
SSSHPIFHRGEFSVCDSVSVWVGDKTTATDIKGKEVMVLGEVNINNSVFKQYFFETKCRDPNPVDSGCRGIDSKHWNSYCTTTHTFVKALTMDGKQAAWRFIRIDTACVCVLSFKAVRRA

SEQ ID NO: 19 - protein, 120 aa, Homo sapiens NGF mutant Arg114Gly
SSSHPIFHRGEFSVCDSVSVWVGDKTTATDIKGKEVMVLGEVNINNSVFKQYFFETKCRDPNPVDSGCRGIDSKHWNSYCTTTHTFVKALTMDGKQAAWRFIRIDTACVCVLSGKAVRRA

SEQ ID NO: 20 - protein, 120 aa, Homo sapiens NGF mutant Arg114Leu
SSSHPIFHRGEFSVCDSVSVWVGDKTTATDIKGKEVMVLGEVNINNSVFKQYFFETKCRDPNPVDSGCRGIDSKHWNSYCTTTHTFVKALTMDGKQAAWRFIRIDTACVCVLSLKAVRRA

SEQ ID NO: 21 - protein, 120 aa, Homo sapiens NGF mutant Phe101Ala
SSSHPIFHRGEFSVCDSVSVWVGDKTTATDIKGKEVMVLGEVNINNSVFKQYFFETKCRDPNPVDSGCRGIDSKHWNSYCTTTHTFVKALTMDGKQAAWRAIRIDTACVCVLSRKAVRRA

SEQ ID NO: 22 - DNA, 726 bp, Encoding gene of Homo sapiens NGF mutant Phe12Glu
atgtccatgttgttctacactctgatcacagcttttctgatcggcatacaggcggaaccacactcagagagcaatgtccctgcaggacacaccatcccccaagcccactggactaaacttcagcattcccttgacactgcccttcgcagagcccgcagcgccccggcagcggcgatagctgcacgcgtggcggggcagacccgcaacattactgtggaccccaggctgtttaaaaagcggcgactccgttcaccccgtgtgctgtttagcacccagcctccccgtgaagctgcagacactcaggatctggacttcgaggtcggtggtgctgcccccttcaacaggactcacaggagcaagcggtcatcatcccatcccatcttccacaggggcgaagagtcggtgtgtgacagtgtcagcgtgtgggttggggataagaccaccgccacagacatcaagggcaaggaggtgatggtgttgggagaggtgaacattaacaacagtgtattcaaacagtacttttttgagaccaagtgccgggacccaaatcccgttgacagcgggtgccggggcattgactcaaagcactggaactcatattgtaccacgactcacacctttgtcaaggcgctgaccatggatggcaagcaggctgcctggcggtttatccggatagatacggcctgtgtgtgtgtgctcagcaggaaggctgtgagaagagcctga

SEQ ID NO: 23 - DNA, 726 bp, Encoding gene of Homo sapiens NGF mutant Lys32Gly
atgtccatgttgttctacactctgatcacagcttttctgatcggcatacaggcggaaccacactcagagagcaatgtccctgcaggacacaccatcccccaagcccactggactaaacttcagcattcccttgacactgcccttcgcagagcccgcagcgccccggcagcggcgatagctgcacgcgtggcggggcagacccgcaacattactgtggaccccaggctgtttaaaaagcggcgactccgttcaccccgtgtgctgtttagcacccagcctccccgtgaagctgcagacactcaggatctggacttcgaggtcggtggtgctgcccccttcaacaggactcacaggagcaagcggtcatcatcccatcccatcttccacaggggcgaattctcggtgtgtgacagtgtcagcgtgtgggttggggataagaccaccgccacagacatcgggggcaaggaggtgatggtgttgggagaggtgaacattaacaacagtgtattcaaacagtacttttttgagaccaagtgccgggacccaaatcccgttgacagcgggtgccggggcattgactcaaagcactggaactcatattgtaccacgactcacacctttgtcaaggcgctgaccatggatggcaagcaggctgcctggcggtttatccggatagatacggcctgtgtgtgtgtgctcagcaggaaggctgtgagaagagcctga

SEQ ID NO: 24 - DNA, 726 bp, Encoding gene of Homo sapiens NGF mutant Lys32Leu
atgtccatgttgttctacactctgatcacagcttttctgatcggcatacaggcggaaccacactcagagagcaatgtccctgcaggacacaccatcccccaagcccactggactaaacttcagcattcccttgacactgcccttcgcagagcccgcagcgccccggcagcggcgatagctgcacgcgtggcggggcagacccgcaacattactgtggaccccaggctgtttaaaaagcggcgactccgttcaccccgtgtgctgtttagcacccagcctccccgtgaagctgcagacactcaggatctggacttcgaggtcggtggtgctgcccccttcaacaggactcacaggagcaagcggtcatcatcccatcccatcttccacaggggcgaattctcggtgtgtgacagtgtcagcgtgtgggttggggataagaccaccgccacagacatcctgggcaaggaggtgatggtgttgggagaggtgaacattaacaacagtgtattcaaacagtacttttttgagaccaagtgccgggacccaaatcccgttgacagcgggtgccggggcattgactcaaagcactggaactcatattgtaccacgactcacacctttgtcaaggcgctgaccatggatggcaagcaggctgcctggcggtttatccggatagatacggcctgtgtgtgtgtgctcagcaggaaggctgtgagaagagcctga

SEQ ID NO: 25 - DNA, 726 bp, Encoding gene of Homo sapiens NGF mutant Lys32Tyr
atgtccatgttgttctacactctgatcacagcttttctgatcggcatacaggcggaaccacactcagagagcaatgtccctgcaggacacaccatcccccaagcccactggactaaacttcagcattcccttgacactgcccttcgcagagcccgcagcgccccggcagcggcgatagctgcacgcgtggcggggcagacccgcaacattactgtggaccccaggctgtttaaaaagcggcgactccgttcaccccgtgtgctgtttagcacccagcctccccgtgaagctgcagacactcaggatctggacttcgaggtcggtggtgctgcccccttcaacaggactcacaggagcaagcggtcatcatcccatcccatcttccacaggggcgaattctcggtgtgtgacagtgtcagcgtgtgggttggggataagaccaccgccacagacatctacggcaaggaggtgatggtgttgggagaggtgaacattaacaacagtgtattcaaacagtacttttttgagaccaagtgccgggacccaaatcccgttgacagcgggtgccggggcattgactcaaagcactggaactcatattgtaccacgactcacacctttgtcaaggcgctgaccatggatggcaagcaggctgcctggcggtttatccggatagatacggcctgtgtgtgtgtgctcagcaggaaggctgtgagaagagcctga

SEQ ID NO: 26 - DNA, 726 bp, Encoding gene of Homo sapiens NGF mutant Arg59Leu
atgtccatgttgttctacactctgatcacagcttttctgatcggcatacaggcggaaccacactcagagagcaatgtccctgcaggacacaccatcccccaagcccactggactaaacttcagcattcccttgacactgcccttcgcagagcccgcagcgccccggcagcggcgatagctgcacgcgtggcggggcagacccgcaacattactgtggaccccaggctgtttaaaaagcggcgactccgttcaccccgtgtgctgtttagcacccagcctccccgtgaagctgcagacactcaggatctggacttcgaggtcggtggtgctgcccccttcaacaggactcacaggagcaagcggtcatcatcccatcccatcttccacaggggcgaattctcggtgtgtgacagtgtcagcgtgtgggttggggataagaccaccgccacagacatcaagggcaaggaggtgatggtgttgggagaggtgaacattaacaacagtgtattcaaacagtacttttttgagaccaagtgcctggacccaaatcccgttgacagcgggtgccggggcattgactcaaagcactggaactcatattgtaccacgactcacacctttgtcaaggcgctgaccatggatggcaagcaggctgcctggcggtttatccggatagatacggcctgtgtgtgtgtgctcagcaggaaggctgtgagaagagcctga

SEQ ID NO: 27 - DNA, 726 bp, Encoding gene of Homo sapiens NGF mutant Arg59Ala
atgtccatgttgttctacactctgatcacagcttttctgatcggcatacaggcggaaccacactcagagagcaatgtccctgcaggacacaccatcccccaagcccactggactaaacttcagcattcccttgacactgcccttcgcagagcccgcagcgccccggcagcggcgatagctgcacgcgtggcggggcagacccgcaacattactgtggaccccaggctgtttaaaaagcggcgactccgttcaccccgtgtgctgtttagcacccagcctccccgtgaagctgcagacactcaggatctggacttcgaggtcggtggtgctgcccccttcaacaggactcacaggagcaagcggtcatcatcccatcccatcttccacaggggcgaattctcggtgtgtgacagtgtcagcgtgtgggttggggataagaccaccgccacagacatcaagggcaaggaggtgatggtgttgggagaggtgaacattaacaacagtgtattcaaacagtacttttttgagaccaagtgcgcggacccaaatcccgttgacagcgggtgccggggcattgactcaaagcactggaactcatattgtaccacgactcacacctttgtcaaggcgctgaccatggatggcaagcaggctgcctggcggtttatccggatagatacggcctgtgtgtgtgtgctcagcaggaaggctgtgagaagagcctga

SEQ ID NO: 28 - DNA, 726 bp, Encoding gene of Homo sapiens NGF mutant Asp65Ala
atgtccatgttgttctacactctgatcacagcttttctgatcggcatacaggcggaaccacactcagagagcaatgtccctgcaggacacaccatcccccaagcccactggactaaacttcagcattcccttgacactgcccttcgcagagcccgcagcgccccggcagcggcgatagctgcacgcgtggcggggcagacccgcaacattactgtggaccccaggctgtttaaaaagcggcgactccgttcaccccgtgtgctgtttagcacccagcctccccgtgaagctgcagacactcaggatctggacttcgaggtcggtggtgctgcccccttcaacaggactcacaggagcaagcggtcatcatcccatcccatcttccacaggggcgaattctcggtgtgtgacagtgtcagcgtgtgggttggggataagaccaccgccacagacatcaagggcaaggaggtgatggtgttgggagaggtgaacattaacaacagtgtattcaaacagtacttttttgagaccaagtgccgggacccaaatcccgttgccagcgggtgccggggcattgactcaaagcactggaactcatattgtaccacgactcacacctttgtcaaggcgctgaccatggatggcaagcaggctgcctggcggtttatccggatagatacggcctgtgtgtgtgtgctcagcaggaaggctgtgagaagagcctga

SEQ ID NO: 29 - DNA, 726 bp, Encoding gene of Homo sapiens NGF mutant Asp65Gly
atgtccatgttgttctacactctgatcacagcttttctgatcggcatacaggcggaaccacactcagagagcaatgtccctgcaggacacaccatcccccaagcccactggactaaacttcagcattcccttgacactgcccttcgcagagcccgcagcgccccggcagcggcgatagctgcacgcgtggcggggcagacccgcaacattactgtggaccccaggctgtttaaaaagcggcgactccgttcaccccgtgtgctgtttagcacccagcctccccgtgaagctgcagacactcaggatctggacttcgaggtcggtggtgctgcccccttcaacaggactcacaggagcaagcggtcatcatcccatcccatcttccacaggggcgaattctcggtgtgtgacagtgtcagcgtgtgggttggggataagaccaccgccacagacatcaagggcaaggaggtgatggtgttgggagaggtgaacattaacaacagtgtattcaaacagtacttttttgagaccaagtgccgggacccaaatcccgttggcagcgggtgccggggcattgactcaaagcactggaactcatattgtaccacgactcacacctttgtcaaggcgctgaccatggatggcaagcaggctgcctggcggtttatccggatagatacggcctgtgtgtgtgtgctcagcaggaaggctgtgagaagagcctga

SEQ ID NO: 30 - DNA, 726 bp, Encoding gene of Homo sapiens NGF mutant Lys74Leu
atgtccatgttgttctacactctgatcacagcttttctgatcggcatacaggcggaaccacactcagagagcaatgtccctgcaggacacaccatcccccaagcccactggactaaacttcagcattcccttgacactgcccttcgcagagcccgcagcgccccggcagcggcgatagctgcacgcgtggcggggcagacccgcaacattactgtggaccccaggctgtttaaaaagcggcgactccgttcaccccgtgtgctgtttagcacccagcctccccgtgaagctgcagacactcaggatctggacttcgaggtcggtggtgctgcccccttcaacaggactcacaggagcaagcggtcatcatcccatcccatcttccacaggggcgaattctcggtgtgtgacagtgtcagcgtgtgggttggggataagaccaccgccacagacatcaagggcaaggaggtgatggtgttgggagaggtgaacattaacaacagtgtattcaaacagtacttttttgagaccaagtgccgggacccaaatcccgttgacagcgggtgccggggcattgactcattgcactggaactcatattgtaccacgactcacacctttgtcaaggcgctgaccatggatggcaagcaggctgcctggcggtttatccggatagatacggcctgtgtgtgtgtgctcagcaggaaggctgtgagaagagcctga

SEQ ID NO: 31 - DNA, 726 bp, Encoding gene of Homo sapiens NGF mutant Lys88Phe
atgtccatgttgttctacactctgatcacagcttttctgatcggcatacaggcggaaccacactcagagagcaatgtccctgcaggacacaccatcccccaagcccactggactaaacttcagcattcccttgacactgcccttcgcagagcccgcagcgccccggcagcggcgatagctgcacgcgtggcggggcagacccgcaacattactgtggaccccaggctgtttaaaaagcggcgactccgttcaccccgtgtgctgtttagcacccagcctccccgtgaagctgcagacactcaggatctggacttcgaggtcggtggtgctgcccccttcaacaggactcacaggagcaagcggtcatcatcccatcccatcttccacaggggcgaattctcggtgtgtgacagtgtcagcgtgtgggttggggataagaccaccgccacagacatcaagggcaaggaggtgatggtgttgggagaggtgaacattaacaacagtgtattcaaacagtacttttttgagaccaagtgccgggacccaaatcccgttgacagcgggtgccggggcattgactcaaagcactggaactcatattgtaccacgactcacacctttgtctttgcgctgaccatggatggcaagcaggctgcctggcggtttatccggatagatacggcctgtgtgtgtgtgctcagcaggaaggctgtgagaagagcctga

SEQ ID NO: 32 - DNA, 726 bp, Encoding gene of Homo sapiens NGF mutant Lys88Leu
atgtccatgttgttctacactctgatcacagcttttctgatcggcatacaggcggaaccacactcagagagcaatgtccctgcaggacacaccatcccccaagcccactggactaaacttcagcattcccttgacactgcccttcgcagagcccgcagcgccccggcagcggcgatagctgcacgcgtggcggggcagacccgcaacattactgtggaccccaggctgtttaaaaagcggcgactccgttcaccccgtgtgctgtttagcacccagcctccccgtgaagctgcagacactcaggatctggacttcgaggtcggtggtgctgcccccttcaacaggactcacaggagcaagcggtcatcatcccatcccatcttccacaggggcgaattctcggtgtgtgacagtgtcagcgtgtgggttggggataagaccaccgccacagacatcaagggcaaggaggtgatggtgttgggagaggtgaacattaacaacagtgtattcaaacagtacttttttgagaccaagtgccgggacccaaatcccgttgacagcgggtgccggggcattgactcaaagcactggaactcatattgtaccacgactcacacctttgtcttggcgctgaccatggatggcaagcaggctgcctggcggtttatccggatagatacggcctgtgtgtgtgtgctcagcaggaaggctgtgagaagagcctga

SEQ ID NO: 33 - DNA, 726 bp, Encoding gene of Homo sapiens NGF mutant Lys88Glu
atgtccatgttgttctacactctgatcacagcttttctgatcggcatacaggcggaaccacactcagagagcaatgtccctgcaggacacaccatcccccaagcccactggactaaacttcagcattcccttgacactgcccttcgcagagcccgcagcgccccggcagcggcgatagctgcacgcgtggcggggcagacccgcaacattactgtggaccccaggctgtttaaaaagcggcgactccgttcaccccgtgtgctgtttagcacccagcctccccgtgaagctgcagacactcaggatctggacttcgaggtcggtggtgctgcccccttcaacaggactcacaggagcaagcggtcatcatcccatcccatcttccacaggggcgaattctcggtgtgtgacagtgtcagcgtgtgggttggggataagaccaccgccacagacatcaagggcaaggaggtgatggtgttgggagaggtgaacattaacaacagtgtattcaaacagtacttttttgagaccaagtgccgggacccaaatcccgttgacagcgggtgccggggcattgactcaaagcactggaactcatattgtaccacgactcacacctttgtcgaggcgctgaccatggatggcaagcaggctgcctggcggtttatccggatagatacggcctgtgtgtgtgtgctcagcaggaaggctgtgagaagagcctga

SEQ ID NO: 34 - DNA, 726 bp, Encoding gene of Homo sapiens NGF mutant Lys88Gly
atgtccatgttgttctacactctgatcacagcttttctgatcggcatacaggcggaaccacactcagagagcaatgtccctgcaggacacaccatcccccaagcccactggactaaacttcagcattcccttgacactgcccttcgcagagcccgcagcgccccggcagcggcgatagctgcacgcgtggcggggcagacccgcaacattactgtggaccccaggctgtttaaaaagcggcgactccgttcaccccgtgtgctgtttagcacccagcctccccgtgaagctgcagacactcaggatctggacttcgaggtcggtggtgctgcccccttcaacaggactcacaggagcaagcggtcatcatcccatcccatcttccacaggggcgaattctcggtgtgtgacagtgtcagcgtgtgggttggggataagaccaccgccacagacatcaagggcaaggaggtgatggtgttgggagaggtgaacattaacaacagtgtattcaaacagtacttttttgagaccaagtgccgggacccaaatcccgttgacagcgggtgccggggcattgactcaaagcactggaactcatattgtaccacgactcacacctttgtcggggcgctgaccatggatggcaagcaggctgcctggcggtttatccggatagatacggcctgtgtgtgtgtgctcagcaggaaggctgtgagaagagcctga

SEQ ID NO: 35 - DNA, 726 bp, Encoding gene of Homo sapiens NGF mutant Gln96Glu
atgtccatgttgttctacactctgatcacagcttttctgatcggcatacaggcggaaccacactcagagagcaatgtccctgcaggacacaccatcccccaagcccactggactaaacttcagcattcccttgacactgcccttcgcagagcccgcagcgccccggcagcggcgatagctgcacgcgtggcggggcagacccgcaacattactgtggaccccaggctgtttaaaaagcggcgactccgttcaccccgtgtgctgtttagcacccagcctccccgtgaagctgcagacactcaggatctggacttcgaggtcggtggtgctgcccccttcaacaggactcacaggagcaagcggtcatcatcccatcccatcttccacaggggcgaattctcggtgtgtgacagtgtcagcgtgtgggttggggataagaccaccgccacagacatcaagggcaaggaggtgatggtgttgggagaggtgaacattaacaacagtgtattcaaacagtacttttttgagaccaagtgccgggacccaaatcccgttgacagcgggtgccggggcattgactcaaagcactggaactcatattgtaccacgactcacacctttgtcaaggcgctgaccatggatggcaaggaggctgcctggcggtttatccggatagatacggcctgtgtgtgtgtgctcagcaggaaggctgtgagaagagcctga

SEQ ID NO: 36 - DNA, 726 bp, Encoding gene of Homo sapiens NGF mutant Arg114Val
atgtccatgttgttctacactctgatcacagcttttctgatcggcatacaggcggaaccacactcagagagcaatgtccctgcaggacacaccatcccccaagcccactggactaaacttcagcattcccttgacactgcccttcgcagagcccgcagcgccccggcagcggcgatagctgcacgcgtggcggggcagacccgcaacattactgtggaccccaggctgtttaaaaagcggcgactccgttcaccccgtgtgctgtttagcacccagcctccccgtgaagctgcagacactcaggatctggacttcgaggtcggtggtgctgcccccttcaacaggactcacaggagcaagcggtcatcatcccatcccatcttccacaggggcgaattctcggtgtgtgacagtgtcagcgtgtgggttggggataagaccaccgccacagacatcaagggcaaggaggtgatggtgttgggagaggtgaacattaacaacagtgtattcaaacagtacttttttgagaccaagtgccgggacccaaatcccgttgacagcgggtgccggggcattgactcaaagcactggaactcatattgtaccacgactcacacctttgtcaaggcgctgaccatggatggcaagcaggctgcctggcggtttatccggatagatacggcctgtgtgtgtgtgctcagcgtcaaggctgtgagaagagcctga

SEQ ID NO: 37 - DNA, 726 bp, Encoding gene of Homo sapiens NGF mutant Arg114Phe
atgtccatgttgttctacactctgatcacagcttttctgatcggcatacaggcggaaccacactcagagagcaatgtccctgcaggacacaccatcccccaagcccactggactaaacttcagcattcccttgacactgcccttcgcagagcccgcagcgccccggcagcggcgatagctgcacgcgtggcggggcagacccgcaacattactgtggaccccaggctgtttaaaaagcggcgactccgttcaccccgtgtgctgtttagcacccagcctccccgtgaagctgcagacactcaggatctggacttcgaggtcggtggtgctgcccccttcaacaggactcacaggagcaagcggtcatcatcccatcccatcttccacaggggcgaattctcggtgtgtgacagtgtcagcgtgtgggttggggataagaccaccgccacagacatcaagggcaaggaggtgatggtgttgggagaggtgaacattaacaacagtgtattcaaacagtacttttttgagaccaagtgccgggacccaaatcccgttgacagcgggtgccggggcattgactcaaagcactggaactcatattgtaccacgactcacacctttgtcaaggcgctgaccatggatggcaagcaggctgcctggcggtttatccggatagatacggcctgtgtgtgtgtgctcagcttcaaggctgtgagaagagcctga

SEQ ID NO: 38 - DNA, 726 bp, Encoding gene of Homo sapiens NGF mutant Arg114Gly
atgtccatgttgttctacactctgatcacagcttttctgatcggcatacaggcggaaccacactcagagagcaatgtccctgcaggacacaccatcccccaagcccactggactaaacttcagcattcccttgacactgcccttcgcagagcccgcagcgccccggcagcggcgatagctgcacgcgtggcggggcagacccgcaacattactgtggaccccaggctgtttaaaaagcggcgactccgttcaccccgtgtgctgtttagcacccagcctccccgtgaagctgcagacactcaggatctggacttcgaggtcggtggtgctgcccccttcaacaggactcacaggagcaagcggtcatcatcccatcccatcttccacaggggcgaattctcggtgtgtgacagtgtcagcgtgtgggttggggataagaccaccgccacagacatcaagggcaaggaggtgatggtgttgggagaggtgaacattaacaacagtgtattcaaacagtacttttttgagaccaagtgccgggacccaaatcccgttgacagcgggtgccggggcattgactcaaagcactggaactcatattgtaccacgactcacacctttgtcaaggcgctgaccatggatggcaagcaggctgcctggcggtttatccggatagatacggcctgtgtgtgtgtgctcagcgggaaggctgtgagaagagcctga

SEQ ID NO: 39 - DNA, 726 bp, Encoding gene of Homo sapiens NGF mutant Arg114Leu
atgtccatgttgttctacactctgatcacagcttttctgatcggcatacaggcggaaccacactcagagagcaatgtccctgcaggacacaccatcccccaagcccactggactaaacttcagcattcccttgacactgcccttcgcagagcccgcagcgccccggcagcggcgatagctgcacgcgtggcggggcagacccgcaacattactgtggaccccaggctgtttaaaaagcggcgactccgttcaccccgtgtgctgtttagcacccagcctccccgtgaagctgcagacactcaggatctggacttcgaggtcggtggtgctgcccccttcaacaggactcacaggagcaagcggtcatcatcccatcccatcttccacaggggcgaattctcggtgtgtgacagtgtcagcgtgtgggttggggataagaccaccgccacagacatcaagggcaaggaggtgatggtgttgggagaggtgaacattaacaacagtgtattcaaacagtacttttttgagaccaagtgccgggacccaaatcccgttgacagcgggtgccggggcattgactcaaagcactggaactcatattgtaccacgactcacacctttgtcaaggcgctgaccatggatggcaagcaggctgcctggcggtttatccggatagatacggcctgtgtgtgtgtgctcagcttgaaggctgtgagaagagcctga

SEQ ID NO: 40 - DNA, 726 bp, Encoding gene of Homo sapiens NGF mutant Phe101Ala
atgtccatgttgttctacactctgatcacagcttttctgatcggcatacaggcggaaccacactcagagagcaatgtccctgcaggacacaccatcccccaagcccactggactaaacttcagcattcccttgacactgcccttcgcagagcccgcagcgccccggcagcggcgatagctgcacgcgtggcggggcagacccgcaacattactgtggaccccaggctgtttaaaaagcggcgactccgttcaccccgtgtgctgtttagcacccagcctccccgtgaagctgcagacactcaggatctggacttcgaggtcggtggtgctgcccccttcaacaggactcacaggagcaagcggtcatcatcccatcccatcttccacaggggcgaattctcggtgtgtgacagtgtcagcgtgtgggttggggataagaccaccgccacagacatcaagggcaaggaggtgatggtgttgggagaggtgaacattaacaacagtgtattcaaacagtacttttttgagaccaagtgccgggacccaaatcccgttgacagcgggtgccggggcattgactcaaagcactggaactcatattgtaccacgactcacacctttgtcaaggcgctgaccatggatggcaagcaggctgcctggcgggcgatccggatagatacggcctgtgtgtgtgtgctcagcaggaaggctgtgagaagagcctga

SEQ ID NO: 41 - DNA, 19 bp, Artificial primer F sequence
ggaattcatgtccatgttg

SEQ ID NO: 42 - DNA, 19 bp, Artificial primer R sequence
caagctttcaggctcttct